European Patent Specification EP 3 423 489 B1, published August 7, 2024. Title: ANTIBODIES TO CD40 WITH ENHANCED AGONIST ACTIVITY. Applicant: The Rockefeller University. The sequence listing filed with the application follows.

SEQUENCE LISTING (13 sequences)

SEQ ID NO: 1 - protein, 456 aa, Homo sapiens
QVQLVQSGAEVKKPGASVKVSCKASGYTFTGYYMHWVRQAPGQGLEWMGWINPDSGGTNYAQKFQGRVTMTRDTSISTAYMELNRLRSDDTAVYYCARDQPLGYCTNGVCSYFDYWGQGTLVTVSSATTKGPSVFPLAPSSKSTSGGTAALGCLVKDYFPEPVTVSWNSGALTSGVHTFPAVLQSSGLYSLSSVVTVPSSSLGTQTYICNVNHKPSNTKVDKRVEPKSCDKTHTCPPCPAPELLGGPSVFLFPPKPKDTLMISRTPEVTCVVVDVSHEDPEVKFNWYVDGVEVHNAKTKPREEQYNSTYRVVSVLTVLHQDWLNGKEYKCKVSNKALPAPIEKTISKAKGQPREPQVYTLPPSRDELTKNQVSLTCLVKGFYPSDIAVEWESNGQPENNYKTTPPVLDSDGSFFLYSKLTVDKSRWQQGNVFSCSVMHEALHNHYTQKSLSLSPGK

SEQ ID NO: 2 - protein, 214 aa, Homo sapiens
DIQMTQSPSSVSASVGDRVTITCRASQGIYSWLAWYQQKPGKAPNLLIYTASTLQSGVPSRFSGSGSGTDFTLTISSLQPEDFATYYCQQANIFPLTFGGGTKVEIKRTVAAPSVFIFPPSDEQLKSGTASVVCLLNNFYPREAKVQWKVDNALQSGNSQESVTEQDSKDSTYSLSSTLTLSKADYEKHKVYACEVTHQGLSSPVTKSFNRGEC

SEQ ID NO: 3 - protein, 456 aa, Artificial Sequence
  synthetic sequence
QVQLVQSGAEVKKPGASVKVSCKASGYTFTGYYMHWVRQAPGQGLEWMGWINPDSGGTNYAQKFQGRVTMTRDTSISTAYMELNRLRSDDTAVYYCARDQPLGYCTNGVCSYFDYWGQGTLVTVSSATTKGPSVFPLAPSSKSTSGGTAALGCLVKDYFPEPVTVSWNSGALTSGVHTFPAVLQSSGLYSLSSVVTVPSSSLGTQTYICNVNHKPSNTKVDKRVEPKSCDKTHTCPPCPAPELLGGPSVFLFPPKPKDTLMISRTPEVTCVVVDVSHEDPEVKFNWYVDGVEVHNAKTKPREEQYASTYRVVSVLTVLHQDWLNGKEYKCKVSNKALPAPIEKTISKAKGQPREPQVYTLPPSRDELTKNQVSLTCLVKGFYPSDIAVEWESNGQPENNYKTTPPVLDSDGSFFLYSKLTVDKSRWQQGNVFSCSVMHEALHNHYTQKSLSLSPGK

SEQ ID NO: 4 - protein, 456 aa, Artificial Sequence
  synthetic sequence
QVQLVQSGAEVKKPGASVKVSCKASGYTFTGYYMHWVRQAPGQGLEWMGWINPDSGGTNYAQKFQGRVTMTRDTSISTAYMELNRLRSDDTAVYYCARDQPLGYCTNGVCSYFDYWGQGTLVTVSSATTKGPSVFPLAPSSKSTSGGTAALGCLVKDYFPEPVTVSWNSGALTSGVHTFPAVLQSSGLYSLSSVVTVPSSSLGTQTYICNVNHKPSNTKVDKRVEPKSCDKTHTCPPCPAPELLGGPSVFLFPPKPKDTLMISRTPEVTCVVVDVEHEDPEVKFNWYVDGVEVHNAKTKPREEQYNSTYRVVSVLTVLHQDWLNGKEYKCKVSNKALPAPIEKTISKAKGQPREPQVYTLPPSRDELTKNQVSLTCLVKGFYPSDIAVEWESNGQPENNYKTTPPVLDSDGSFFLYSKLTVDKSRWQQGNVFSCSVMHEALHNHYTQKSLSLSPGK

SEQ ID NO: 5 - protein, 456 aa, Artificial Sequence
  synthetic sequence
QVQLVQSGAEVKKPGASVKVSCKASGYTFTGYYMHWVRQAPGQGLEWMGWINPDSGGTNYAQKFQGRVTMTRDTSISTAYMELNRLRSDDTAVYYCARDQPLGYCTNGVCSYFDYWGQGTLVTVSSATTKGPSVFPLAPSSKSTSGGTAALGCLVKDYFPEPVTVSWNSGALTSGVHTFPAVLQSSGLYSLSSVVTVPSSSLGTQTYICNVNHKPSNTKVDKRVEPKSCDKTHTCPPCPAPELLGGPSVFLFPPKPKDTLMISRTPEVTCVVVDVEHEDPEVKFNWYVDGVEVHNAKTKPREEQYNSTYRVVSVLTVLHQDWLNGKEYKCKVSNKAFPAPIEKTISKAKGQPREPQVYTLPPSRDELTKNQVSLTCLVKGFYPSDIAVEWESNGQPENNYKTTPPVLDSDGSFFLYSKLTVDKSRWQQGNVFSCSVMHEALHNHYTQKSLSLSPGK

SEQ ID NO: 6 - protein, 456 aa, Artificial Sequence
  synthetic sequence
QVQLVQSGAEVKKPGASVKVSCKASGYTFTGYYMHWVRQAPGQGLEWMGWINPDSGGTNYAQKFQGRVTMTRDTSISTAYMELNRLRSDDTAVYYCARDQPLGYCTNGVCSYFDYWGQGTLVTVSSATTKGPSVFPLAPSSKSTSGGTAALGCLVKDYFPEPVTVSWNSGALTSGVHTFPAVLQSSGLYSLSSVVTVPSSSLGTQTYICNVNHKPSNTKVDKRVEPKSCDKTHTCPPCPAPELLGDDSVFLFPPKPKDTLMISRTPEVTCVVVDVSHEDGEVKFNWYVDGVEVHNAKTKPREEQYNSTYRVVSVLTVLHQDWLNGKEYKCKVSNKALPRPIEKTISKAKGQPREPQVYTLPPSRDELTKNQVSLTCLVKGFYPSDIAVEWESNGQPENNYKTTPPVLDSDGSFFLYSKLTVDKSRWQQGNVFSCSVMHEALHNHYTQKSLSLSPGK

SEQ ID NO: 7 - protein, 456 aa, Artificial Sequence
  synthetic sequence
QVQLVQSGAEVKKPGASVKVSCKASGYTFTGYYMHWVRQAPGQGLEWMGWINPDSGGTNYAQKFQGRVTMTRDTSISTAYMELNRLRSDDTAVYYCARDQPLGYCTNGVCSYFDYWGQGTLVTVSSATTKGPSVFPLAPSSKSTSGGTAALGCLVKDYFPEPVTVSWNSGALTSGVHTFPAVLQSSGLYSLSSVVTVPSSSLGTQTYICNVNHKPSNTKVDKRVEPKSCDKTHTCPPCPAPELLGDDSVFLFPPKPKDTLMISRTPEVTCVVVDVSDEDGEVKFNWYVDGVEVHNAKTKPREEQYNSTYRVVSVLTVLHQDWLNGKEYKCKVSNKALPRPIEKTISKAKGQPREPQVYTLPPSRDELTKNQVSLTCLVKGFYPSDIAVEWESNGQPENNYKTTPPVLDSDGSFFLYSKLTVDKSRWQQGNVFSCSVMHEALHNHYTQKSLSLSPGK

SEQ ID NO: 8 - protein, 452 aa, Homo sapiens
QVQLVQSGAEVKKPGASVKVSCKASGYTFTGYYMHWVRQAPGQGLEWMGWINPDSGGTNYAQKFQGRVTMTRDTSISTAYMELNRLRSDDTAVYYCARDQPLGYCTNGVCSYFDYWGQGTLVTVSSASTKGPSVFPLAPCSRSTSESTAALGCLVKDYFPEPVTVSWNSGALTSGVHTFPAVLQSSGLYSLSSVVTVPSSNFGTQTYTCNVDHKPSNTKVDKTVERKCCVECPPCPAPPVAGPSVFLFPPKPKDTLMISRTPEVTCVVVDVSHEDPEVQFNWYVDGVEVHNAKTKPREEQFNSTFRVVSVLTVVHQDWLNGKEYKCKVSNKGLPAPIEKTISKTKGQPREPQVYTLPPSREEMTKNQVSLTCLVKGFYPSDIAVEWESNGQPENNYKTTPPMLDSDGSFFLYSKLTVDKSRWQQGNVFSCSVMHEALHNHYTQKSLSLSPGK

SEQ ID NO: 9 - protein, 452 aa, Artificial Sequence
  synthetic sequence
QVQLVQSGAEVKKPGASVKVSCKASGYTFTGYYMHWVRQAPGQGLEWMGWINPDSGGTNYAQKFQGRVTMTRDTSISTAYMELNRLRSDDTAVYYCARDQPLGYCTNGVCSYFDYWGQGTLVTVSSASTKGPSVFPLAPSSRSTSESTAALGCLVKDYFPEPVTVSWNSGALTSGVHTFPAVLQSSGLYSLSSVVTVPSSNFGTQTYTCNVDHKPSNTKVDKTVERKCCVECPPCPAPPVAGPSVFLFPPKPKDTLMISRTPEVTCVVVDVSHEDPEVQFNWYVDGVEVHNAKTKPREEQFNSTFRVVSVLTVVHQDWLNGKEYKCKVSNKGLPAPIEKTISKTKGQPREPQVYTLPPSREEMTKNQVSLTCLVKGFYPSDIAVEWESNGQPENNYKTTPPMLDSDGSFFLYSKLTVDKSRWQQGNVFSCSVMHEALHNHYTQKSLSLSPGK

SEQ ID NO: 10 - protein, 452 aa, Artificial Sequence
  synthetic sequence
QVQLVQSGAEVKKPGASVKVSCKASGYTFTGYYMHWVRQAPGQGLEWMGWINPDSGGTNYAQKFQGRVTMTRDTSISTAYMELNRLRSDDTAVYYCARDQPLGYCTNGVCSYFDYWGQGTLVTVSSASTKGPSVFPLAPCSRSTSESTAALGCLVKDYFPEPVTVSWNSGALTSGVHTFPAVLQSSGLYSLSSVVTVPSSNFGTQTYTCNVDHKPSNTKVDKTVERKSCVECPPCPAPPVAGPSVFLFPPKPKDTLMISRTPEVTCVVVDVSHEDPEVQFNWYVDGVEVHNAKTKPREEQFNSTFRVVSVLTVVHQDWLNGKEYKCKVSNKGLPAPIEKTISKTKGQPREPQVYTLPPSREEMTKNQVSLTCLVKGFYPSDIAVEWESNGQPENNYKTTPPMLDSDGSFFLYSKLTVDKSRWQQGNVFSCSVMHEALHNHYTQKSLSLSPGK

SEQ ID NO: 11 - protein, 277 aa, Homo sapiens
MVRLPLQCVLWGCLLTAVHPEPPTACREKQYLINSQCCSLCQPGQKLVSDCTEFTETECLPCGESEFLDTWNRETHCHQHKYCDPNLGLRVQQKGTSETDTICTCEEGWHCTSEACESCVLHRSCSPGFGVKQIATGVSDTICEPCPVGFFSNVSSAFEKCHPWTSCETKDLVVQQAGTNKTDVVCGPQDRLRALVVIPIIFGILFAILLVLVFIKKVAKKPTNKAPHPKQEPQEINFPDDLPGSNTAAPVQETLHGCQPVTQEDGKESRISVQERQ

SEQ ID NO: 12 - protein, 261 aa, Homo sapiens
MIETYNQTSPRSAATGLPISMKIFMYLLTVFLITQMIGSALFAVYLHRRLDKIEDERNLHEDFVFMKTIQRCNTGERSLSLLNCEEIKSQFEGFVKDIMLNKEETKKENSFEMQKGDQNPQIAAHVISEASSKTTSVLQWAEKGYYTMSNNLVTLENGKQLTVKRQGLYYIYAQVTFCSNREASSQAPFIASLCLKSPGRFERILLRAANTHSSAKPCGQQSIHLGGVFELQPGASVFVNVTDPSQVSHGTGFTSFGLLKL

SEQ ID NO: 13 - protein, 20 aa, Homo sapiens
MVRLPLQCVLWGCLLTAVHP